European Patent Specification EP 3 663 406 B1, published February 26, 2025. Title: Biological processes for the production of aryl sulfates. Applicant: CysBio ApS. The sequence listing filed with the application follows.

SEQUENCE LISTING (75 sequences)

SEQ ID NO: 1 - protein, 291 aa, Rattus norvegicus
MEFSRPPLVHVKGIPLIKYFAETIGPLQNFTAWPDDLLISTYPKSGTTWMSEILDMIYQGGKLEKCGRAPIYARVPFLEFKCPGVPSGLETLEETPAPRLLKTHLPLSLLPQSLLDQKVKVIYIARNAKDVVVSYYNFYNMAKLHPDPGTWDSFLENFMDGEVSYGSWYQHVKEWWELRHTHPVLYLFYEDIKENPKREIKKILEFLGRSLPEETVDSIVHHTSFKKMKENCMTNYTTIPTEIMDHNVSPFMRKGTTGDWKNTFTVAQNERFDAHYAKTMTDCDFKFRCEL

SEQ ID NO: 2 - protein, 295 aa, Homo sapiens [sequence omitted]

SEQ ID NO: 3 - protein, 295 aa, Equus caballus
MELIQDTSRPPLKYVKGVPLIKYFAEALGPLQSFQARPDDLLISTYPKSGTTWVSEILDMIYHGGDLEKCRRAPIFIRVPFLEFKAPEIPSGVEVLKDTPAPRLLKTHLPLSLLPQTLLDQKVKVVYLARNAKDVAVSYYHFYRMAKVHPDPGTWDSFLEKFMAGEVSYGSWYKHVQEWWELSHTHPVLYLFYEDMKENPKKEIQKILEFVGRSLPEETLDRIVQHTSFKEMKKNPMANYSTIPCDIMDHNISAFMRKGIAGDWKNTFTVAQNEHFDTDYAEKMAGCKLSFRSEV

SEQ ID NO: 4 - protein, 295 aa, Sus scrofa
MEPVQDTYRPPLEYVKGVPLIKYFAEALGPLESFQAWPDDVLISTYPKSGTTWVSEILDLIYQGGDLQKCQRAPIFVRVPFLEFKIPGCPTGFELLKDTPAPRLLKTHLPLALLPQTLLDQKVKVVYVARNAKDVAVSYYHFYRMAKVHPNPGTWDSFLEDFMAGEVSYGSWYQHVQEWWELRHTHPVLYLFYEDMKENPKREIQKILEFVGRSLPEETVEDIVQHTSFQEMKNNAMTNYRTLPSDLLDHSISAFMRKGITGDWKSTFTVAQNERFEADYAEKMAGCNLRFRSEL

SEQ ID NO: 5 - protein, 295 aa, Canis lupus
MEDIPDTSRPPLKYVKGIPLIKYFAEALESLQDFQAQPDDLLISTYPKSGTTWVSEILDMIYQDGDVEKCRRAPVFIRVPFLEFKAPGIPTGLEVLKDTPAPRLIKTHLPLALLPQTLLDQKVKVVYVARNAKDVAVSYYHFYRMAKVHPDPDTWDSFLEKFMAGEVSYGSWYQHVQEWWELSHTHPVLYLFYEDMKENPKREIQKILKFVGRSLPEETVDLIVQHTSFKEMKNNSMANYTTLSPDIMDHSISAFMRKGISGDWKTTFTVAQNERFDADYAKKMEGCGLSFRTQL

SEQ ID NO: 6 - protein, 294 aa, Gallus gallus
MGNDEVIRQDLGCLYDIPLYKCFVAGWPQVEAFQARPDDLLIATYPKSGTTWLSEILDAIYHDGDLEKCRRDAIYNRVPFLEMKAPGILSGVEQLEKIPSPRLVKTHLPVHLLPASFQEKDCKVIYMARNAKDVVISYYYFYQMAKIHPDPGTLSEFLQAFMDGKVAYGSWYKHVKGWWEKRHEKRLLYLFYEDMKKDPRREIQKILQFLGKEVAEETVARILHHTSFQEMKKNPATNYETMPTELMDHSLSPFMRKGISGDWANHFTVAQNERFDQHYQQQMAGSDLCFQMEA

SEQ ID NO: 7 - protein, 307 aa, Gallus gallus
MALDKMENLSLEENMLRSEMGEVQGIPVTKPTCDIWDQVWNFKARPDDLLVATYAKAGTTWTQEIVDMIQQNGDIEKCRRASTYKRHPFLEWYIPDSSPLGYSGLKLAEAMPSPRTMKTHLPVQLVPPSFWEQNCKIIYVARNAKDNLVSYYHFHRMNKVLPDPGTIEEFTEKFMNGEVLWGSWYDHVKGWWKAKDKHRILYLFYEDMKENPKREIQKIMKFLEKDLDEEVLNKIIYNTSFEIMKDNPMTNYTKDFVGVMDHSVSPFMRKGSVGDWKNYFTVALNKKFDQDYKKKMADTSLVFRMEL

SEQ ID NO: 8 - protein, 301 aa, Danio rerio
MDLPDISSIKLPSRPKIFEFEGISMISYFTDNWEKLKNFQARPDDILIATYPKAGTTWVSYILDLLYFGKVEPNGQSSLPIYMRVPFLESCFPGMPSGTELADNLPNSPRLIKTHLPVQLVPKSFWGQNSKVVYVARNAKDNVVSFFHFDRMNHGQPEPGDWDTFLQAFIKGERVFGSWFDHVCGWWEKKKTYPNLHYMFYEDIAKDINGEVESLCTFLKLSRSDEEKEKIINGVQFDAMKQNVMTNYSTIPTMDFTISPFMRKGKVGDWKNHFTVAQNEQFDEDYKEKMKNTTLNFRTKI

SEQ ID NO: 9 - protein, 300 aa, Danio rerio
MEIQGKSSTDLPDRPEIFEFEGISMVEHFTKNWENVKNFQARPDDILIATYPKAGTTWVSNILDLLYFGKEDPKRQTTKPIYKRVPFLESCFPEMQSGTELANNLPTSPRLIKTHLPVQLVPQSFWEKNSRVAYVARNAKDNAVSYFHFNRMNKAQPEPGDWNTFLEEFMKGKMVFGSWFDHVCGWWEKKKTYPNLHYMLYEDMAKDIKGEVESLCTFLKLSRSDEEKEKIINGIQFDAMKQNKMTNYSTVLVMDFTISPFMRKGKVGDWKNHFTVAQNEQFNEDYKQKMKNSTLKFPTE

SEQ ID NO: 10 - protein, 338 aa, Drosophila melanogaster
MPQSSFFAKSVPFEQIDKLAISGGYSSIFASSKPSVPVVGNWEQRFCRLADTFQPVLDRVYDFEVRDDDVWIVTLPKCGTTWMQELAWLVINECDFETAKSVDLTHRSPFLEFNGVVPNVPHDTIAAANALPSPRLIKSHLPAWMLPRQIWSKRPKIIYVYRNPKDAAISYFHHWRGMVGYQGTKSDFMHSFIDGYVNFTPCWPHILDFWQLRHEPNIFFTSYERMKGQLGQVISEVAQFLERSVSQEQMQQMQRHLSFESMRDNPACNHVKEFESMKAAAGREVEEFRFVRRGVVGSHKDELTADIIREFDLWSDSNLRDFKLNMDDFANYSKFAST

SEQ ID NO: 11 - protein, 313 aa, Drosophila melanogaster
MNRVQVTPRSYPTNLIDKDWGNRKLFYTKDSENFLRLVHDMKLRDDDVWIVTLPKCGTTWMQELLWLLLNNCDFEGALAKDQELRTPFLEFGYSVFHDPNRSFGPIEDLKSPRLIKSHLSLALLPSKLWEGKNKVIYVSRNPLDSYVSRYYHGVSFGFNYGKSLHQYFDEVLASDDFPTEFIEHAHEFYQLRNEPWVFYTSFEMMKKDLRGVINDVSRFLNKPINDQQMEKLLKHLSFAEMKKNPTTNHLWELAQVQHENAGKEMHPFVRRGDVNGYKDELKPEQIEKANVRIQEVLAKNGVTLDELLLLKDQ

SEQ ID NO: 12 - protein, 346 aa, Drosophila melanogaster
MENTPLKFPHEIRDVEESTNAELLDHFHGERTGFVQVGSEGYFFPHKYKDEAERYYNFEARPDDVWIATVPRSGTTWTQELIWLVANGLDFEHAQERPLTERFPFFEFPLFVHPKIKEELQEENRDSAEALEFIEKIARPGYEALSEIPRSQRRFIKTHFPFSLMPPSVLEKKCKVIYVVRDPKDVAVSYYHLNRLFRTQGYVGDFERYWHYFQNGLNPWLPYYSHVKEAREHAHLSNVLFLRYEDMLADLPGAINSIASFLECPPKPEDMDRLLDHLSIRSFRENKSVNMHEMASVGVLNKGEAGFVRSGAKTAYQPQQEFVENPKLLKSANEWVEQNIKSFKTI

SEQ ID NO: 13 - protein, 323 aa, Arabidopsis thaliana
MEMNLRIEDLNEETKTLISSLPSDKDFTGKTICKYQGCWYTHNVLQAVLNFQKSFKPQDTDIIVASFPKCGTTWLKALTFALLHRSKQPSHDDDHPLLSNNPHVLVPYFEIDLYLRSENPDLTKFSSSPRLFSTHVPSHTLQEGLKGSTCKIVYISRNVKDTLVSYWHFFTKKQTDEKIISSFEDTFEMFCRGVSIFGPFWDHVLSYWRGSLEDPNHVLFMKFEEMKAEPRDQIKKFAEFLGCPFTKEEEESGSVDEIIDLCSLRNLSSLEINKTGKLNSGRENKMFFRKGEVGDWKNYLTPEMENKIDMIIQEKLQNSGLKF

SEQ ID NO: 14 - protein, 506 aa, Flavobacterium johnsoniae
MNTINEYLSLEEFEAIIFGNQKVTISDVVVNRVNESFNFLKEFSGNKVIYGVNTGFGPMAQYRIKESDQIQLQYNLIRSHSSGTGKPLSPVCAKAAILARLNTLSLGNSGVHPSVINLMSELINKDITPLIFEHGGVGASGDLVQLSHLALVLIGEGEVFYKGERRPTPEVFEIEGLKPIQVEIREGLALINGTSVMTGIGVVNVYHAKKLLDWSLKSSCAINELVQAYDDHFSAELNQTKRHKGQQEIALKMRQNLSDSTLIRKREDHLYSGENTEEIFKEKVQEYYSLRCVPQILGPVLETINNVASILEDEFNSANDNPIIDVKNQHVYHGGNFHGDYISLEMDKLKIVITKLTMLAERQLNYLLNSKINELLPPFVNLGTLGFNFGMQGVQFTATSTTAESQMLSNPMYVHSIPNNNDNQDIVSMGTNSAVITSKVIENAFEVLAIEMITIVQAIDYLGQKDKISSVSKKWYDEIRNIIPTFKEDQVMYPFVQKVKDHLINN

SEQ ID NO: 15 - protein, 552 aa, Herpetosiphon aurantiacus
MSTTLILTGEGLGIDDVVRVARHQDRVELTTDPAILAQIEASCAYINQAVKEHQPVYGVTTGFGGMANVIISPEEAAELQNNAIWYHKTGAGKLLPFTDVRAAMLLRANSHMRGASGIRLEIIQRMVTFLNANVTPHVREFGSIGASGDLVPLISITGALLGTDQAFMVDFNGETLDCISALERLGLPRLRLQPKEGLAMMNGTSVMTGIAANCVHDARILLALALEAHALMIQGLQGTNQSFHPFIHRHKPHTGQVWAADHMLELLQGSQLSRNELDGSHDYRDGDLIQDRYSLRCLPQFLGPIIDGMAFISHHLRVEINSANDNPLIDTASAASYHGGNFLGQYIGVGMDQLRYYMGLMAKHLDVQIALLVSPQFNNGLPASLVGNIQRKVNMGLKGLQLTANSIMPILTFLGNSLADRFPTHAEQFNQNINSQGFGSANLARQTIQTLQQYIAITLMFGVQAVDLRTHKLAGHYNAAELLSPLTAKIYHAVRSIVKHPPSPERPYIWNDDEQVLEAHISALAHDIANDGSLVSAVEQTLSGLRSIILFR

SEQ ID NO: 16 - protein, 552 aa, Herpetosiphon aurantiacus
MRHQVTLTGAGLTIEDVVRVARHHQPVGLTDNPEILQRIEDSCAYINDAVKASKPVYGVTTGFGGMADVVISSEEAADLQNNAIWYHKTGAGKLLPLADVRAAMLLRANSHMRGVSGIRLEIIQRMMTFLNANVTPHVREFGSIGASGDLVPLISITGALLGTDPAFRVDFDGENIDCLEALERLNLPRLELLPKEGLAMMNGTSVMTGIASNVLHDARILLGLALNIHGLMIQGLQGTNQSFHPFIHQHKAHTGQVWAADHMLQILEGSALSRDELDGRHEYREGDLIQDRYSLRCLPQFLGPIIDGMAYITHHLRVEINSANDNPLINTEAGASYHGGNFLGQYIGVGMDQLRYYMGLMAKHLDVQIALLVSPQFNNGLSASLVGNTDRKVNMGLKGLQISGNSIMPILGFLGNSLADRFPTHAEQFNQNINSQGFGSANLARQTIETLQQYIAIALIFGVQAVDLRTFKRTGHYNAVETLSPMTAKLYSAMREVVGKPISHERPYIWNDNEQALEQHISAIVSDITNDGIIPQAIQETLDSLRSIILFA

SEQ ID NO: 17 - protein, 523 aa, Rhodobacter sphaeroides
MLAMSPPKPAVELDRHIDLDEAHSVASGGARIVLAPPARDRCRASEARLGAVIREARHVYGLTTGFGPLANRLVSGENVRTLQANLVHHLASGVGPVLDWTTARAMVLARLVAIAQGASGASEGTIARLIDLLNSELAPAVPMRGTVGASGDLTPLAHMVLCLQGRGDFLDRDGTRLDGAEGLRRGRLQPLDLSHRDALALVNGTSAMTGIALVNAHACRHLGNWAVALTALLAECLGGRTEAWAAALSDLRPHPGQKDAAARLRARVDGSARVVRHVIAERRLGASDIGTEPEAGQDAYSLRCAPQVLGAGFDTLAWHDRVLTIELNAVTDNPVFPPDGSVPALHGGNFMGQHVALTSDALATAVTVLAGLAERQIARLTDERLNRGLPPFLHRGPAGLNSGFMGAQVTATALLAEMRATGPASIHSISTNAANQDVVSLGTIAARLCREKIDRWAEILAILALCLAQAAELRCGSGLDGVSPAGKKLVQALREQFPPLETDRPLGQEIAALATHLLQQSPV

SEQ ID NO: 18 - protein, 510 aa, Saccharothrix espanaensis
MTQVVERQADRLSSREYLARVVRSAGWDAGLTSCTDEEIVRMGASARTIEEYLKSDKPIYGLTQGFGPLVLFDADSELEQGGSLISHLGTGQGAPLAPEVSRLILWLRIQNMRKGYSAVSPVFWQKLADLWNKGFTPAIPRHGTVSASGDLQPLAHAALAFTGVGEAWTRDADGRWSTVPAVDALAALGAEPFDWPVREALAFVNGTGASLAVAVLNHRSALRLVRACAVLSARLATLLGANPEHYDVGHGVARGQVGQLTAAEWIRQGLPRGMVRDGSRPLQEPYSLRCAPQVLGAVLDQLDGAGDVLAREVDGCQDNPITYEGELLHGGNFHAMPVGFASDQIGLAMHMAAYLAERQLGLLVSPVTNGDLPPMLTPRAGRGAGLAGVQISATSFVSRIRQLVFPASLTTLPTNGWNQDHVPMALNGANSVFEALELGWLTVGSLAVGVAQLAAMTGHAAEGVWAELAGICPPLDADRPLGAEVRAARDLLSAHADQLLVDEADGKDFG

SEQ ID NO: 19 - protein, 519 aa, Rheinheimera sp. A13L
MRSEQLTLEDVEAIALGRQTLVVTEKQMHAVENAHKFLCRAISDRKRIYGVTTGYGPLATTEVDPRQSALLQQNLVHHLCSGVGDPLTHPQVRAMMVARLISLLSGHSGANPLLIKRMQEWLDADIVPFIPCRGTVGASGDLTPLAHLARALSGGGKVSIKGGLWIESRDAHQQLGWQPLVLKGKDAISLVNGTSATVGIAALNATAAERALKLSTLLVLLYAELLNGHREAFHPAIGQLRPHPGQQKLHSWLWSLSASSDALVPWCAESRNLNLMGEDIQQNQPLLQDAYTLRCAPQALGAALDVISQHATTVKIELSAVTDNPLLFAEDELILHGGNFFGQHLAFASDHLNNALIQMALYSERRIARITDPLRNKGLPAFMQPLDTGLHSGFMGAQVCATSLVAELRSQAMPASIQSIPTNADNQDIVPLGTIAARRASTSLTQLYQILAIEALVLVQGAELKNTHSFSHSSQVVCAWLRQYALPLKEDRALSEDITRVAEALIDPDKVKSLIELLA

SEQ ID NO: 20 - protein, 713 aa, Rhodotorula mucilaginosa
MAPSVDSIATSVANSLSNGLHAAAAANGGDVHKKTAGAGSLLPTTETTQLDIVERILADAGATDQIKLDGYTLTLGDVVGAARRGRSVKVADSPHIREKIDASVEFLRTQLDNSVYGVTTGFGGSADTRTEDAISLQKALLEHQLCGVLPTSMDGFALGRGLENSLPLEVVRGAMTIRVNSLTRGHSAVRIVVLEALTNFLNHGITPIVPLRGTISASGDLSPLSYIAASITGHPDSKVHVDGKIMSAQEAIALKGLQPVVLGPKEGLGLVNGTAVSASMATLALTDAHVLSLLAQALTALTVEAMVGHAGSFHPFLHDVTRPHPTQIEVARNIRTLLEGSKYAVHHETEVKVKDDEGILRQDRYPLRCSPQWLGPLVSDMIHAHAVLSLEAGQSTTDNPLIDLENKMTHHGGAFMASSVGNTMEKTRLAVALMGKVSFTQLTEMLNAGMNRALPSCLAAEDPSLSYHCKGLDIAAAAYTSELGHLANPVSTHVQPAEMGNQAINSLALISARRTAEANDVLSLLLATHLYCVLQAVDLRAMEFEHTKAFEPMVTELLKQHFGALATAEVEDKVRKSIYKRLQQNNSYDLEQRWHDTFSVATGAVVEALAGQEVSLASLNAWKVACAEKAIALTRSVRDSFWAAPSSSSPALKYLSPRTRVLYSFVREEVGVKARRGDVYLGKQEVTIGTNVSRIYEAIKSGCIAPVLVKMMA

SEQ ID NO: 21 - protein, 689 aa, Trichosporon cutaneum
MFIETNVAKPASTKAMNAGSAKAAPVEPFATYAHSQATKTVSIDGHTMKVGDVVAVARHGAKVELAASVAGPVRASVDFKESKKHTSIYGVTTGFGGSADTRTSDTEALQISLLEHQLCGFLPTDATYEGMLLAAMPIPIVRGAMAVRVNSCVRGHSGVRLEVLQSFADFINRGLVPCVPLRGTISASGDLSPLSYIAGAICGHPDVKVFDTAASPPTVLTSPEAIAKYGLKTVKLASKEGLGLVNGTAVSAAAGALALYDAECLAIMSQTNTVLTVEALDGHVGSFAPFIQEIRPHAGQIEAARNIRHMLGGSKLAVHEESELLADQDAGILRQDRYALRTSAQWIGPQLEALGLARQQIETELNSTTDNPLIDVEGGMFHHGGNFQAMAVTSAMDSARIVLQNLGKLSFAQVTELINCEMNHGLPSNLAGSEPSTNYHCKGLDIHCGAYCAELGFLANPMSNHVQSTEMHNQSVNSMAFASARRTMEANEVLSLLLGSQMYCATQALDLRVMEVKFKMAIVKLLNETLTKHFAAFLTPEQLAKLNTHAAITLYKRLNQTPSWDSAPRFEDAAKHLVGVIMDALMVNDDITDLTNLPKWKKEFAKEAGNLYRSILVATTADGRNDLEPAEYLGQTRAVYEAVRSELGVKVRRGDVAEGKSGKSIGSSVAKIVEAMRDGRLMGAVGKMF

SEQ ID NO: 22 - protein, 716 aa, Rhodosporidium toruloides
MAPSLDSISHSFANGVASAKQAVNGASTNLAVAGSHLPTTQVTQVDIVEKMLAAPTDSTLELDGYSLNLGDVVSAARKGRPVRVKDSDEIRSKIDKSVEFLRSQLSMSVYGVTTGFGGSADTRTEDAISLQKALLEHQLCGVLPSSFDSFRLGRGLENSLPLEVVRGAMTIRVNSLTRGHSAVRLVVLEALTNFLNHGITPIVPLRGTISASGDLSPLSYIAAAISGHPDSKVHVVHEGKEKILYAREAMALFNLEPVVLGPKEGLGLVNGTAVSASMATLALHDAHMLSLLSQSLTAMTVEAMVGHAGSFHPFLHDVTRPHPTQIEVAGNIRKLLEGSRFAVHHEEEVKVKDDEGILRQDRYPLRTSPQWLGPLVSDLIHAHAVLTIEAGQSTTDNPLIDVENKTSHHGGNFQAAAVANTMEKTRLGLAQIGKLNFTQLTEMLNAGMNRGLPSCLAAEDPSLSYHCKGLDIAAAAYTSELGHLANPVTTHVQPAEMANQAVNSLALISARRTTESNDVLSLLLATHLYCVLQAIDLRAIEFEFKKQFGPAIVSLIDQHFGSAMTGSNLRDELVEKVNKTLAKRLEQTNSYDLVPRWHDAFSFAAGTVVEVLSSTSLSLAAVNAWKVAAAESAISLTRQVRETFWSAASTSSPALSYLSPRTQILYAFVREELGVKARRGDVFLGKQEVTIGSNVSKIYEAIKSGRINNVLLKMLA

SEQ ID NO: 23 - protein, 737 aa, Phanerochaete chrysosporium
MPSRIDYYTSSGNGYAQSRKSSAIYPASASTGHAAPSTERKPELLDKFVEAYDELQSYREGKPVIVDGHNLSIPAVAATARFGAAVVLDENPETHERVLQSRRVIVDKVSTQRSVYGVSTGFGGSADTRTSDPLQLGHALLQHQHVGVLPTQTESPLPALPLGDPLATTSMPEAWVRGAILIRMNSLIRGHSGVRWELIEKMGELLRENITPLVPLRGSISASGDLSPLSYIAGTLIGSPAIRVFDGPASYGARRILPSNIALANHGVAPIPLSSKEHLGILNGTAFSASVGALALNEAVHLSLLAQVCTAMGTEAMIGAVGSFDAFIHDTARPHPGQVEVARNVRTLLEDSQMAVKAEDEVHIAEDEGELRQDRYPLRTAAQFLGPQIEDILSAHETVTLECNSTTDNPLIDGETGTVHHGGNFQAMAVTNAMEKTRLAIHHIGKLLFAQATELINPMMNRGLPPNLAATDPSHNYFAKGVDIHLAAYVGELGFLASPVSSHIQSAEMHNQAVNSLALVSARYTISALDVLSLLTAAYLYVLCQALDLRAMHNDLQSSLSAIVRELLPKHFPSAAKRADALLPILERTIFRALNSSSSADCKARMVSVAASTTTPLVDFLSADAALASELANITAFRTELATRAADALTTLRTQYLEGARGAAPASKYLGKTRPVYEFVRVTLNVPMHGRENLHNFEMGPGVEDGIIGNNISTIYEAIRDGKMQNVVMQLVKSIKA

SEQ ID NO: 24 - protein, 14 aa, Artificial Sequence
  His-Tag
MAHHHHHHENLYFQ

SEQ ID NO: 25 - protein, 302 aa, Escherichia coli
MDQIRLTHLRQLEAESIHIIREVAAEFSNPVMLYSIGKDSSVMLHLARKAFYPGTLPFPLLHVDTGWKFREMYEFRDRTAKAYGCELLVHKNPEGVAMGINPFVHGSAKHTDIMKTEGLKQALNKYGFDAAFGGARRDEEKSRAKERIYSFRDRFHRWDPKNQRPELWHNYNGQINKGESIRVFPLSNWTEQDIWQYIWLENIDIVPLYLAAERPVLERDGMLMMIDDNRIDLQPGEVIKKRMVRFRTLGCWPLTGAVESNAQTLPEIIEEMLVSTTSERQGRVIDRDQAGSMELKKRQGYF

SEQ ID NO: 26 - protein, 475 aa, Escherichia coli
MNTALAQQIANEGGVEAWMIAQQHKSLLRFLTCGSVDDGKSTLIGRLLHDTRQIYEDQLSSLHNDSKRHGTQGEKLDLALLVDGLQAEREQGITIDVAYRYFSTEKRKFIIADTPGHEQYTRNMATGASTCELAILLIDARKGVLDQTRRHSFISTLLGIKHLVVAINKMDLVDYSEETFTRIREDYLTFAGQLPGNLDIRFVPLSALEGDNVASQSESMPWYSGPTLLEVLETVEIQRVVDAQPMRFPVQYVNRPNLDFRGYAGTLASGRVEVGQRVKVLPSGVESNVARIVTFDGDREEAFAGEAITLVLTDEIDISRGDLLLAADEALPAVQSASVDVVWMAEQPLSPGQSYDIKIAGKKTRARVDGIRYQVDINNLTQREVENLPLNGIGLVDLTFDEPLVLDRYQQNPVTGGLIFIDRLSNVTVGAGMVHEPVSQATAAPSEFSAFELELNALVRRHFPHWGARDLLGDK

SEQ ID NO: 27 - protein, 201 aa, Escherichia coli
MALHDENVVWHSHPVTVQQRELHHGHRGVVLWFTGLSGSGKSTVAGALEEALHKLGVSTYLLDGDNVRHGLCSDLGFSDADRKENIRRVGEVANLMVEAGLVVLTAFISPHRAERQMVRERVGEGRFIEVFVDTPLAICEARDPKGLYKKARAGELRNFTGIDSVYEAPESAEIHLNGEQLVTNLVQQLLDLLRQNDIIRS

SEQ ID NO: 28 - protein, 246 aa, Escherichia coli
MLDQVCQLARNAGDAIMQVYDGTKPMDVVSKADNSPVTAADIAAHTVIMDGLRTLTPDVPVLSEEDPPGWEVRQHWQRYWLVDPLDGTKEFIKRNGEFTVNIALIDHGKPILGVVYAPVMNVMYSAAEGKAWKEECGVRKQIQVRDARPPLVVISRSHADAELKEYLQQLGEHQTTSIGSSLKFCLVAEGQAQLYPRFGPTNIWDTAAGHAVAAAAGAHVHDWQGKPLDYTPRESFLNPGFRVSIY

SEQ ID NO: 29 - DNA, 58 bp, Artificial Sequence
  Primer CBJP472
tagaaataattttgtttaactttaagaaggagatataccatggagttctcccgtccac

SEQ ID NO: 30 - DNA, 49 bp, Artificial Sequence
  Primer CBJP473
taagcattatgcggccgcaagcttgtcatagttcacaacgaaacttgaa

SEQ ID NO: 31 - DNA, 62 bp, Artificial Sequence
  Primer CBJP470
tagaaataattttgtttaactttaagaaggagatataccatggaactgattcaggataccag

SEQ ID NO: 32 - DNA, 47 bp, Artificial Sequence
  Primer CBJP471
taagcattatgcggccgcaagcttgttacagttcgctacgaaagctc

SEQ ID NO: 33 - DNA, 60 bp, Artificial Sequence
  Primer CBJP499
tagaaataattttgtttaactttaagaaggagatataccatggagctgatccaggacacc

SEQ ID NO: 34 - DNA, 45 bp, Artificial Sequence
  Primer CBJP500
taagcattatgcggccgcaagcttgtcacacctctgagcggaagc

SEQ ID NO: 35 - DNA, 57 bp, Artificial Sequence
  Primer CBJP505
tagaaataattttgtttaactttaagaaggagatataccatggagccggtccaggac

SEQ ID NO: 36 - DNA, 45 bp, Artificial Sequence
  Primer CBJP506
taagcattatgcggccgcaagcttgtcacagctcagagcggaagc

SEQ ID NO: 37 - DNA, 57 bp, Artificial Sequence
  Primer CBJP503
tagaaataattttgtttaactttaagaaggagatataccatggaggacattcccgac

SEQ ID NO: 38 - DNA, 45 bp, Artificial Sequence
  Primer CBJP504
taagcattatgcggccgcaagcttgtcacagctgtgtgcggaagc

SEQ ID NO: 39 - DNA, 62 bp, Artificial Sequence
  Primer CBJP501
tagaaataattttgtttaactttaagaaggagatataccatggggaatgatgaggtgatcag

SEQ ID NO: 40 - DNA, 54 bp, Artificial Sequence
  Primer CBJP502
taagcattatgcggccgcaagcttgttactctgtctattgcaatttattacagg

SEQ ID NO: 41 - DNA, 65 bp, Artificial Sequence
  Primer CBJP491
catcttagtatattagttaagtataagaaggagatatacatatggatcaaatacgacttactcac

SEQ ID NO: 42 - DNA, 46 bp, Artificial Sequence
  Primer CBJP492
tggccggccgatatccaattgatcaggatctgataatatcgttctg

SEQ ID NO: 43 - DNA, 24 bp, Artificial Sequence
  Primer CBJP497
tcaggatctgataatatcgttctg

SEQ ID NO: 44 - DNA, 59 bp, Artificial Sequence
  Primer CBJP498
cagaacgatattatcagatcctgataagttaacaccgctcacagagacgaggtggagaa

SEQ ID NO: 45 - DNA, 46 bp, Artificial Sequence
  Primer CBJP496
tggccggccgatatccaattgattagtaaatagacactctgaaccc

SEQ ID NO: 46 - DNA, 62 bp, Artificial Sequence
  Primer CBJP487
catcttagtatattagttaagtataagaaggagatatacatatggcaccgagcgttgatagc

SEQ ID NO: 47 - DNA, 47 bp, Artificial Sequence
  Primer CBJP488
tggccggccgatatccaattgattaggccatcattttaaccagaacc

SEQ ID NO: 48 - protein, 540 aa, Rhodobacter capsulatus
MLDATIGRKRMTLQSQTAKDCLALDGALTLVQCEAIATHRSRISVTPALRERCARAHARLEHAIAEQRHIYGITTGFGPLANRLIGADQGAELQQNLIYHLATGVGPKLSWAEARALMLARLNSILQGASGASPETIDRIVAVLNAGFAPEVPAQGTVGASGDLTPLAHMVLALQGRGRMIDPSGRVQEAGAVMDRLCGGPLTLAARDGLALVNGTSAMTAIAALTGVEAARAIDAALRHSAVLMEVLSGHAEAWHPAFAELRPHPGQLRATERLAQALDGAGRVCRTLTAARRLTAADLRPEDHPAQDAYSLRVVPQLVGAVWDTLDWHDRVVTCELNSVTDNPIFPEGCAVPALHGGNFMGVHVALASDALNAALVTLAGLVERQIARLTDEKLNKGLPAFLHGGQAGLQSGFMGAQVTATALLAEMRANATPVSVQSLSTNGANQDVVSMGTIAARRARAQLLPLSQIQAILALALAQAMDLLDDPEGQAGWSLTARDLRDRIRAVSPGLRADRPLAGDIEAVAQGLRHPSAADPPA

SEQ ID NO: 49 - DNA, 1620 bp, Rhodobacter capsulatus
atgctggatgcaaccattggtcgtaaacgtatgaccctgcagagccagaccgcaaaagattgtctggcactggatggtgcactgaccctggttcagtgtgaagcaattgcaacccatcgtagccgtattagcgttacaccggcactgcgtgaacgttgtgcacgtgcccatgcacgtctggaacatgcaattgccgaacagcgtcatatttatggtattaccaccggttttggtccgctggcaaatcgtctgattggtgcagatcagggtgcagaactgcagcagaatctgatttatcatctggcaaccggtgtgggtccgaaactgagctgggctgaagcccgtgcactgatgctggcacgtctgaatagcatcctgcagggtgcaagcggtgcaagtccggaaaccattgatcgcattgttgccgttctgaatgcaggttttgcaccggaagttccggcacagggcaccgttggtgccagcggtgatctgactccgctggcccatatggttctggccctgcaaggtcgtggtcgtatgattgatccgagcggtcgtgttcaagaggcaggcgcagttatggatcgtctgtgtggcggtccgctgacactggcagcacgtgatggtctggcgctggttaatggcaccagcgcaatgaccgcaattgcagcactgaccggtgttgaagccgcacgtgcaattgatgcagccctgcgtcatagcgcagttctgatggaagttctgagcggtcatgcagaagcatggcatccggcatttgcggaactgcgtccgcatccgggtcagctgcgtgcaaccgaacgtctggcacaggccctggatggcgcaggtcgtgtttgtcgtaccctgaccgcagcacgtcgtctgacagcagccgatctgcgtccggaagatcatcctgcacaggatgcatatagcctgcgtgttgttccgcagctggttggtgcagtttgggataccctggattggcatgatcgtgttgttacctgtgaactgaatagcgttaccgataatccgatttttccggaaggttgtgcagttcctgccctgcatggtggcaattttatgggtgttcatgttgcactggcaagtgatgcactgaatgccgcactggttaccctggcaggtctggttgaacgtcagattgcccgtctgaccgatgaaaaactgaataaaggtctgcctgcctttctgcatggcggtcaggctggtctgcagagcggttttatgggagcacaggttaccgcaaccgcactgctggcagaaatgcgtgcaaatgcgacaccggttagcgttcagagcctgagcaccaatggtgcgaatcaggatgttgttagcatgggtacaattgccgcacgtcgtgcgcgtgcacagctgctgccgctgagccagattcaggcaatcctggccctggctctggcccaggcaatggatctgctggatgatccggaaggccaggcaggttggagtctgaccgcacgtgatctgcgtgatcgtattcgtgcagttagtccgggtctgcgtgcagatcgtcctctggcaggcgatattgaagcagttgcacagggactgcgtcatccgagcgcagcggatcctccggca

SEQ ID NO: 50 - DNA, 1569 bp, Rhodobacter sphaeroides
atgctggcaatgagccctccgaaaccggcagttgaactggatcgtcatattgatctggatgaagcacatagcgttgcaagcggtggtgcacgtattgttctggcaccgcctgcacgtgatcgttgtcgtgcaagcgaagcacgtctgggtgcagttattcgtgaagcccgtcatgtttatggtctgaccaccggttttggtccgctggcaaatcgtctggttagcggtgaaaatgttcgtaccctgcaggcaaatctggttcatcatctggccagcggtgtgggtccggttctggattggaccaccgcacgtgcaatggtgctggcacgcctggttgcaattgcccagggtgcgagcggtgcaagtgaaggtacaattgcacgtctgattgatctgctgaatagcgaactggcaccggcagtgccgatgcgtggcaccgttggtgcatcaggtgatctgactccgctggcccatatggttctgtgtctgcagggtcgtggtgattttctggatcgtgatggcacccgtctggatggtgccgaaggtctgcgtcgtggtcgtctgcagccgctggatctgagccatcgtgatgcactggcactggttaatggcaccagcgcaatgacaggtattgcactggtgaatgcacatgcctgtcgtcatctgggtaattgggcagttgcactgaccgcactgctggccgaatgtctgggtggtcgtaccgaagcatgggcagcagcactgagcgatctgcgtccgcatccgggtcagaaagatgcagcagcccgtctgcgtgcacgtgttgatggtagcgcacgtgtggttcgtcatgttattgcagaacgtcgcctgggtgccagcgatattggcaccgaaccggaagcaggtcaggatgcatatagcctgcgttgtgcaccgcaggttctgggtgccggttttgataccctggcatggcatgatcgtgttctgaccattgaactgaatgcagttaccgataatccggtttttcctccggatggtagtgttccggcactgcatggtggcaattttatgggtcagcatgttgccctgacctcagatgccctggcaaccgcagtgaccgttctggcaggtctggccgaacgtcagattgcccgtctgaccgatgaacgtctgaatcgtggtctgcctccgtttctgcaccgtggtccggcaggcctgaatagtggctttatgggtgcacaggttaccgcaacagccctgctggcagaaatgcgtgcaaccggtccggcaagcattcatagcattagcaccaatgcagcaaatcaggatgttgttagcctgggtacgattgccgcacgtctgtgtcgtgaaaaaattgatcgttgggcagaaattctggccattctggcactgtgtctggcacaggcagcagaactgcgttgcggtagtggcctggatggcgtttcaccggcaggtaaaaaactggttcaggcactgcgcgaacagtttccgcctctggaaaccgatcgtccgctgggtcaagaaattgcagcactggcaacccatctgctgcaacagagtccggtt

SEQ ID NO: 51 - DNA, 1518 bp, Flavobacterium johnsoniae
atgaacaccatcaacgaatatctgagcctggaagaatttgaagccattatctttggcaatcagaaagtgaccattagtgatgttgttgtgaatcgcgttaacgagagctttaactttctgaaagaatttagcggcaacaaagtgatctatggtgtgaataccggttttggtccgatggcacagtatcgtattaaagaaagcgatcagattcagctgcagtataatctgattcgtagccatagcagcggcaccggtaaaccgctgagtccggtttgtgcaaaagcagcaattctggcacgtctgaataccctgagtctgggtaatagcggtgttcatccgagcgttattaatctgatgagcgaactgatcaacaaagatatcacaccgctgatttttgaacatggtggtgttggtgcaagcggtgatctggttcagctgagccatctggcactggttctgattggtgaaggtgaagttttctataaaggtgaacgtcgtccgacaccggaagtttttgaaattgaaggtctgaaaccgatccaggtggaaattcgcgaaggtctggccctgattaatggcaccagcgttatgaccggtattggtgttgttaatgtgtaccatgcaaaaaaactgctggattggagcctgaaaagcagctgtgcaattaatgaactggttcaggcatatgatgatcactttagcgcagaactgaatcagaccaaacgtcataaaggtcagcaagaaattgcactgaaaatgcgtcagaatctgagcgatagcaccctgattcgcaaacgtgaagatcatctgtatagcggtgaaaacaccgaagaaatcttcaaagaaaaagtgcaagagtattatagcctgcgttgtgttccgcagattctgggtccggttctggaaaccattaacaatgttgcaagcattctggaagatgaatttaacagcgcaaacgataacccgatcatcgatgttaaaaaccagcatgtttatcacggtggcaattttcatggtgattatatcagcctggaaatggataaactgaaaatcgtgattaccaaactgaccatgctggcagaacgtcagctgaattatctgctgaatagcaaaattaacgaactgctgcctccgtttgttaatctgggcaccctgggttttaactttggtatgcagggtgttcagtttaccgcaaccagcaccaccgcagaaagccagatgctgagcaatccgatgtatgttcatagcattccgaacaataatgataaccaggatattgttagcatgggcaccaatagcgcagttattaccagcaaagttatcgaaaatgcctttgaagttctggccattgaaatgattaccattgttcaggcgattgattatctgggccagaaagataaaatcagcagcgttagcaaaaaatggtatgatgaaatccgcaacatcatcccgacctttaaagaagatcaggtgatgtatccgttcgtgcagaaagtaaaagaccacctgattaacaat

SEQ ID NO: 52 - DNA, 59 bp, Artificial Sequence
  Primer CBJP483
catcttagtatattagttaagtataagaaggagatatacatatgctggcaatgagccct

SEQ ID NO: 53 - DNA, 41 bp, Artificial Sequence
  Primer CBJP484
tggccggccgatatccaattgattaaaccggactctgttgc

SEQ ID NO: 54 - DNA, 65 bp, Artificial Sequence
  Primer CBJP555
catcttagtatattagttaagtataagaaggagatatacatatgaacaccatcaacgaatatctg

SEQ ID NO: 55 - DNA, 55 bp, Artificial Sequence
  Primer CBJP556
tggccggccgatatccaattgattaattgttaatcaggtggtcttttactttctg

SEQ ID NO: 56 - DNA, 61 bp, Artificial Sequence
  Primer CBJP745
catcttagtatattagttaagtataagaaggagatatacatatgctggatgcaaccattgg

SEQ ID NO: 57 - DNA, 41 bp, Artificial Sequence
  Primer CBJP746
tggccggccgatatccaattgattatgccggaggatccgct

SEQ ID NO: 58 - DNA, 33 bp, Artificial Sequence
  Primer CBJP633
agtgcagguaaaacaatggagttctcccgtcca

SEQ ID NO: 59 - DNA, 30 bp, Artificial Sequence
  Primer CBJP634
cgtgcgautcatagttcacaacgaaacttg

SEQ ID NO: 60 - DNA, 34 bp, Artificial Sequence
  Primer CBJP635
atctgtcauaaaacaatggaattttcacgtccgc

SEQ ID NO: 61 - DNA, 32 bp, Artificial Sequence
  Primer CBJP636
cacgcgautcacagttcacaacgaaatttgaa

SEQ ID NO: 62 - DNA, 25 bp, Artificial Sequence
  Primer PTEF1_fw
cacgcgaugcacacaccatagcttc

SEQ ID NO: 63 - DNA, 25 bp, Artificial Sequence
  Primer PTEF1_rv
cgtgcgauggaagtaccttcaaaga

SEQ ID NO: 64 - DNA, 58 bp, Artificial Sequence
  Primer CBJP517
tagaaataattttgtttaactttaagaaggagatataccatggccctggataaaatgg

SEQ ID NO: 65 - DNA, 49 bp, Artificial Sequence
  Primer CBJP518
taagcattatgcggccgcaagcttgtcacaattccatgcgaaaaactag

SEQ ID NO: 66 - DNA, 56 bp, Artificial Sequence
  Primer CBJP533
tagaaataattttgtttaactttaagaaggagatataccatggaattttcacgtcc

SEQ ID NO: 67 - DNA, 47 bp, Artificial Sequence
  Primer CBJP534
taagcattatgcggccgcaagcttgttacagttcacaacgaaatttg

SEQ ID NO: 68 - protein, 511 aa, Saccharomyces cerevisiae
MPAPHGGILQDLIARDALKKNELLSEAQSSDILVWNLTPRQLCDIELILNGGFSPLTGFLNENDYSSVVTDSRLADGTLWTIPITLDVDEAFANQIKPDTRIALFQDDEIPIAILTVQDVYKPNKTIEAEKVFRGDPEHPAISYLFNVAGDYYVGGSLEAIQLPQHYDYPGLRKTPAQLRLEFQSRQWDRVVAFQTRNPMHRAHRELTVRAAREANAKVLIHPVVGLTKPGDIDHHTRVRVYQEIIKRYPNGIAFLSLLPLAMRMSGDREAVWHAIIRKNYGASHFIVGRDHAGPGKNSKGVDFYGPYDAQELVESYKHELDIEVVPFRMVTYLPDEDRYAPIDQIDTTKTRTLNISGTELRRRLRVGGEIPEWFSYPEVVKILRESNPPRPKQGFSIVLGNSLTVSREQLSIALLSTFLQFGGGRYYKIFEHNNKTELLSLIQDFIGSGSGLIIPNQWEDDKDSVVGKQNVYLLDTSSSADIQLESADEPISHIVQKVVLFLEDNGFFVF

SEQ ID NO: 69 - protein, 202 aa, Saccharomyces cerevisiae
MATNITWHPNLTYDERKALRKQDGCTIWLTGLSASGKSTIACALEQLLLQKNLSAYRLDGDNIRFGLNKDLGFSEKDRNENIRRISEVSKLFADSCAISITSFISPYRVDRDRARELHKEAGLKFIEIFVDVPLEVAEQRDPKGLYKKAREGVIKEFTGISAPYEAPKAPELHLRTDQKTVEECATIIYEYLISEKIIRKHL

SEQ ID NO: 70 - protein, 357 aa, Saccharomyces cerevisiae
MALERELLVATQAVRKASLLTKRIQSEVISHKDSTTITKNDNSPVTTGDYAAQTIIINAIKSNFPDDKVVGEESSSGLSDAFVSGILNEIKANDEVYNKNYKKDDFLFTNDQFPLKSLEDVRQIIDFGNYEGGRKGRFWCLDPIDGTKGFLRGEQFAVCLALIVDGVVQLGCIGCPNLVLSSYGAQDLKGHESFGYIFRAVRGLGAFYSPSSDAESWTKIHVRHLKDTKDMITLEGVEKGHSSHDEQTAIKNKLNISKSLHLDSQAKYCLLALGLADVYLRLPIKLSYQEKIWDHAAGNVIVHEAGGIHTDAMEDVPLDFGNGRTLATKGVIASSGPRELHDLVVSTSCDVIQSRNA

SEQ ID NO: 71 - protein, 581 aa, Rattus norvegicus
MEIPGSLCKKVKLSNNAQNWGMQRATNVTYQAHHVSRNKRGQVVGTRGGFRGCTVWLTGLSGAGKTTVSMALEEYLVCHGIPCYTLDGDNIRQGLNKNLGFSPEDREENVRRIAEVAKLFADAGLVCITSFISPYTQVRQGFTGIDSEYEKPEAPELVLKTDSCDVNDCVQQVVELLQERDIVPVDASYEVKELYVPENKLHLAKTDAEALPALKINKVDMQWVQVLAEGWATPLNGFMREREYLQCLHFDCLLDGGVINLSVPIVLTATQEDKERLDGCTAFALVYEGRRVAILRNPEFFEHRKEERCARQWGTTCRSHPYIKMILEQGDWLIGGDLQVLDRIYWNDGLDQYRLTPAELKQKFKDMNADAVFAFQLRNPVHNGHALLMQDTHKQLLERGYRRPVLLLHPLGGWTKDDDVPLMWRMKQHAAVLEEGILNPETTVVAIFPSPMMYAGPTEVQWHCRARMVAGANFYIVGRDPAGMPHPETGKDLYEPTHGAKVLTMAPGLITLEIVPFRVAAYNKKKKRMDYYDSDHHEDFEFISGTRMRKLAREGQKPPEGFMAPKAWTVLVEYYKSLEKA

SEQ ID NO: 72 - protein, 614 aa, Rattus norvegicus
MSEIKKQKTDQQKSTNVVYQAHHVSRNKRGQVVGTRGGFRGCTVWLTGLSGAGKTTISFALEEYLVSHAIPCYSLDGDNVRHGLNKNLGFSAGDREENIRRIAEVAKLFADAGLVCITSFISPFAKDRENARKIHESAGLPFFEIFVDAPLNICESRDVKGLYKRARAGEIKGFTGIDSNYEKPETPECVLKTNLSSVSDCVQQVVELLQEQSIVPHTTIKGIHELFVPENKIDQIRAELETLPSLPITKLDLQWVQILSEGWATPLKGFMREKEYLQTLHFDTLLDDGVINMSIPIVLPVSGDDKARLEGCSKFALMYEGRRVALLQDPEFYEHRKEERCSRVWGTASAKHPHIKMVMEGGDWLVGGDLQVLERIRWNDGLDQYRLTPLELKQKCKDMDADAVFAFQLRNPVHNGHALLMQDTRRRLLERGYKHPVLLLHPLGGWTKDDDVPLDWRMKQHAAVLEEGILDPKSTIVAIFPSPMLYAGPTEVQWHCRCRMIAGANFYIVGRDPAGMPHPETKKDLYEPTHGGKVLSMAPGLTSVEIIPFRVAAYNKIKKAMDFYDPARHDEFDFISGTRMRKLAREGEDPPDGFMAPKAWKVLTDYYRSLEKIN

SEQ ID NO: 73 - protein, 389 aa, Bacillus subtilis
MNGNEPHGGVLINRCDPACHFEGCACQAELDQLALSDLELIAIGGYSPLTGFLGEKDYHSVVKEMRLANGLPWSLPITLPVGEKTARQLSAGDHVKLVKDGVTYGMITVTDIYQPDKTQEALSVFKTNDPAHPGVKKLLARPDYYIGGPITVSSLPDKSFEQFYATPAETRAAFQKLGWKTIVGFQTRNPVHRAHEYIQKTALETVDGLLLHPLVGETKSDDIPSDIRMESYQALLNHYYPKDRVMLSVFPAAMRYAGPREAIFHALVRKNYGCTHFIVGRDHAGVGSYYGTYDAQNIFQSFTEEELGIKPLFFEHSFYCRKCGNMGTSKTCPHSPRDHIHLSGTKVRELLRQGKKPPKEFSRPEVAAVLIKGLHQQPVAIKQNSGELQ

SEQ ID NO: 74 - protein, 199 aa, Bacillus subtilis
MTHNPNIIWHPAAISKSDRQSLNGHKSCVLWFTGLSGSGKSVLANAVDEKLYRKGIQSYVLDGDNIRHGLNKDLGFQTGDRIENIRRIGEVAKLFVDSGQMILTAFISPFREDRDMVRALFPKGEFFEIYVKCPLHVCEQRDPKGLYKKARNGEIKHFTGIDSPYEAPLSPDFIIESDQTSISDGADLIINALQNRGII

SEQ ID NO: 75 - protein, 313 aa, Bacillus subtilis
MKTELIRTISLYDTIILHRHVRPDPDAYGSQCGLTEILRETYPEKNIFAVGTPEPSLSFLYSLDEVDNETYEGALVIVCDTANQERIDDQRYPSGAKLMKIDHHPNEDPYGDLLWVDTSASSVSEMIYELYLEGKEHGWKLNTKAAELIYAGIVGDTGRFLFPNTTEKTLKYAGELIQYPFSSSELFNQLYETKLNVVKLNGFIFQNVSLSENGAASVFIKKDTLEKFGTTASEASQLVGTLGNISGIRAWVFFVEEDDQIRVRFRSKGPVINGLARKYNGGGHPLASGASIYSWDEADRILADLETLCKEHE